European Patent Specification EP 3 147 358 B1, published December 24, 2025. Title: A method for the production of monomeric form of matrix metalloprotease 7 (MMP-7) from its association. Applicant: THE CHEMO-SERO-THERAPEUTIC RESEARCH INSTITUTE. The sequence listing filed with the application follows.

SEQUENCE LISTING (9 sequences)

SEQ ID NO: 1 - DNA, 27 bp, Artificial
  Primer used for the cloning of a pro-matrix metalloproteinase-7 gene
ccataggtccaagaacaattgtctctg

SEQ ID NO: 2 - DNA, 26 bp, Artificial
  Primer used for the cloning of a pro-matrix metalloproteinase-7 gene
caatccaatgaatgaatgaatggatg

SEQ ID NO: 3 - DNA, 81 bp, Artificial
  Primer used to obtain a DNA fragment consisting of an alkaline phosphatase signal peptide and a pro-matrix metalloproteinase-7
catatgaaacaaagcactattgcactggcactcttaccgttactgtttacccctgtgaccaaggccctgccgctgcctcag

SEQ ID NO: 4 - DNA, 26 bp, Artificial
  Primer used to obtain a DNA fragment consisting of an alkaline phosphatase signal peptide and a pro-matrix metalloproteinase-7
ggatccctatttctttcttgaattac

SEQ ID NO: 5 - DNA, 35 bp, Artificial
  Primer used to obtain a DNA fragment consisting of a modified alkaline phosphatase signal peptide and a pro-matrix metalloproteinase-7
ctgtttacccctgtgaccaaggaactgccgctgcc

SEQ ID NO: 6 - DNA, 33 bp, Artificial
  Primer used to obtain a DNA fragment consisting of a modified alkaline phosphatase signal peptide and a pro-matrix metalloproteinase-7
cttggtcacaggggtaaacagtggcggtaagag

SEQ ID NO: 7 - protein, 7 aa, Artificial
  A DNP-protein of fluorescent substrate used for measuring the activity of MMP-7
PLGLWAR

SEQ ID NO: 8 - protein, 21 aa, Artificial
  Amino acid sequence of a signal peptide of alkaline phosphatase
MKQSTIALALLPLLFTPVTKA

SEQ ID NO: 9 - protein, 7 aa, Artificial
  A MOCAc-protein of fluorescent substrate used for measuring the activity of MMP-7; Xaa=N À-(2,4-dinitrophenyl)-L-2,3-diaminopropionyl
PLGLXAR